European Patent Application EP 4 474 395 A1, published December 11, 2024. Title: Anti-Fas Ligand (FasL) Antibodies in the Treatment of SJS/TEN Diseases. Applicant: PinCell S.r.l. The sequence listing filed with the application follows.

SEQUENCE LISTING (12 sequences)

SEQ ID NO: 1 - protein, 5 aa, synthetic construct
  REGION 1..5: note = CDR H1 (a1)
RHGIT

SEQ ID NO: 2 - protein, 5 aa, synthetic construct
  REGION 1..5: note = CDR H1 (a2)
SHGIS

SEQ ID NO: 3 - protein, 17 aa, synthetic construct
  REGION 1..17: note = CDR H2 (b1)
WINAYNGNTNYAQKVQG

SEQ ID NO: 4 - protein, 17 aa, synthetic construct
  REGION 1..17: note = CDR H2 (b2)
WINAYSGNTNYAQKLQG

SEQ ID NO: 5 - protein, 11 aa, synthetic construct
  REGION 1..11: note = CDR H3 (c1)
ETMVRGVPLDY

SEQ ID NO: 6 - protein, 11 aa, synthetic construct
  REGION 1..11: note = CDR H3 (c2)
ETMVRGVPCDY

SEQ ID NO: 7 - protein, 12 aa, synthetic construct
  REGION 1..12: note = CDR L1 (a3)
RASQSVSSSYLA

SEQ ID NO: 8 - protein, 7 aa, synthetic construct
  REGION 1..7: note = CDR L2 (b3)
GASSRAT

SEQ ID NO: 9 - protein, 9 aa, synthetic construct
  REGION 1..9: note = CDR L3 (c3)
QQYGSSPWT

SEQ ID NO: 10 - protein, 120 aa, synthetic construct
  REGION 1..120: note = VL region
EIVLTQSPGTLSLSPGERATLSCRASQSVSSSYLAWYQQKPGQAPRLLIYGASSRATGIPDRFSGSGSGTDFTLTISRLEPEDFAVYYCQQYGSSPWTFGQGTKVEIKRTVAAPSVFIFP

SEQ ID NO: 11 - protein, 132 aa, synthetic construct
  REGION 1..132: note = VH region
QVQLVQSGAEVKKPGASVKVSCKASGYIFIRHGITWVRQAPGQGLEWMGWINAYNGNTNYAQKVQGRVTMTTDKSTSTAYMELRSLRSDDAAVYYCARETMVRGVPLDYWGQGTLVTVSSASTKGPSVFPLA

SEQ ID NO: 12 - protein, 132 aa, synthetic construct
  REGION 1..132: note = VH region
QVQLVQSGAEVKKPGASVKVSCKASGYIFISHGISWVRQAPGQGLEWMGWINAYSGNTNYAQKLQGRVTMTTDRSTSTAYMELRSLRSDDTAVYYCARETMVRGVPCDYWGQGTLVTVSSASTKGPSVFPLA